European Patent Application EP 4 534 649 A1, published April 9, 2025. Title: A method of validating as pharmaceutically active a batch of undifferentiated adult stem cells having the potential to differentiate along the hepatic lineage. Applicant: Unicyte AG. The sequence listing filed with the application follows.

SEQUENCE LISTING (22 sequences)

SEQ ID NO: 1 - DNA, 22 bp, synthetic construct
  source 1..22: mol_type = other DNA
actgattctcgatgggttggag

SEQ ID NO: 2 - DNA, 22 bp, synthetic construct
  source 1..22: mol_type = other DNA
tgtttccagcacatgcaaagac

SEQ ID NO: 3 - DNA, 22 bp, synthetic construct
  source 1..22: mol_type = other DNA
tgtttccagcacatgcaaagac

SEQ ID NO: 4 - DNA, 22 bp, synthetic construct
  source 1..22: mol_type = other DNA
atcaagagtggtgtcatggcaa

SEQ ID NO: 5 - DNA, 21 bp, synthetic construct
  source 1..21: mol_type = other DNA
acaactggccgaagaatagca

SEQ ID NO: 6 - DNA, 18 bp, synthetic construct
  source 1..18: mol_type = other DNA
ggttcccagtcgggttca

SEQ ID NO: 7 - DNA, 17 bp, synthetic construct
  source 1..17: mol_type = other DNA
agcaggagtcggggtgg

SEQ ID NO: 8 - DNA, 22 bp, synthetic construct
  source 1..22: mol_type = other DNA
agagctttgatgtcctgggact

SEQ ID NO: 9 - DNA, 16 bp, synthetic construct
  source 1..16: mol_type = other DNA
tgcgagcgctgcacat

SEQ ID NO: 10 - DNA, 24 bp, synthetic construct
  source 1..24: mol_type = other DNA
gcagcgtgtacttatccttcttca

SEQ ID NO: 11 - DNA, 21 bp, synthetic construct
  source 1..21: mol_type = other DNA
ccataaccaagagctcatgcc

SEQ ID NO: 12 - DNA, 18 bp, synthetic construct
  source 1..18: mol_type = other DNA
gggccacgatcgtcttcc

SEQ ID NO: 13 - DNA, 21 bp, synthetic construct
  source 1..21: mol_type = other DNA
cagcgactctgaggaggaaca

SEQ ID NO: 14 - DNA, 19 bp, synthetic construct
  source 1..19: mol_type = other DNA
tgaggaggtttgctgtggc

SEQ ID NO: 15 - DNA, 20 bp, synthetic construct
  source 1..20: mol_type = other DNA
tgtgcacaggagccaagagt

SEQ ID NO: 16 - DNA, 21 bp, synthetic construct
  source 1..21: mol_type = other DNA
attttcttgctgccagtctgg

SEQ ID NO: 17 - DNA, 21 bp, synthetic construct
  source 1..21: mol_type = other DNA
ctgtggacgcaagatttcctc

SEQ ID NO: 18 - DNA, 21 bp, synthetic construct
  source 1..21: mol_type = other DNA
aggatgggaagccatgttctt

SEQ ID NO: 19 - DNA, 21 bp, synthetic construct
  source 1..21: mol_type = other DNA
agtcctgtgaaccagcagtgc

SEQ ID NO: 20 - DNA, 23 bp, synthetic construct
  source 1..23: mol_type = other DNA
gggtgctttgagtgatgttatcc

SEQ ID NO: 21 - DNA, 21 bp, synthetic construct
  source 1..21: mol_type = other DNA
catcccagtgttctgccattc

SEQ ID NO: 22 - DNA, 21 bp, synthetic construct
  source 1..21: mol_type = other DNA
aggtaaaaaactggcagcgga